European Patent Specification EP 3 995 507 B1, published October 4, 2023. Title: IL-15 AND IL-15R-ALPHA SUSHI DOMAIN BASED MODULOKINES. Applicant: CYTUNE Université de Paris Assistance Publique Hôpitaux de Paris Institut National de la Santé et de la Recherche Médicale (INSERM). Application EP Divisional application based on EP18177685.7. The sequence listing filed with the application follows.

SEQUENCE LISTING (19 sequences)

SEQ ID NO: 1 - protein, 114 aa, artificial sequence
  mammalian interleukin 15 consensus sequence
  MISC_FEATURE (1)..(1): X= N, S, T or I
  MISC_FEATURE (3)..(3): X= V, H, I, Q or E
  MISC_FEATURE (4)..(4): X= N, Y, F or D
  MISC_FEATURE (6)..(6): X= I or R
  MISC_FEATURE (7)..(7): X= S, N, L, Y, K or R
  MISC_FEATURE (10)..(10): X= K, E, R or Q
  MISC_FEATURE (11)..(11): X= K, T or R
  MISC_FEATURE (13)..(13): X= E, D or Q
  MISC_FEATURE (14)..(14): X= D, H, S or N
  MISC_FEATURE (16)..(16): X= I or T
  MISC_FEATURE (17)..(17): X=Q, R or K
  MISC_FEATURE (18)..(18): X= S or F
  MISC_FEATURE (19)..(19): X= M, I or L
  MISC_FEATURE (21)..(21): X= I, V or M
  MISC_FEATURE (23)..(23): X=A or T
  MISC_FEATURE (28)..(28): X=E or D
  MISC_FEATURE (30)..(30): X= D or G
  MISC_FEATURE (31)..(31): X= V, F, A or I
  MISC_FEATURE (34)..(34): X= S, N or R
  MISC_FEATURE (37)..(37): X= V or I
  MISC_FEATURE (39)..(39): X= A or T
  MISC_FEATURE (41)..(41): X= K, Q or N
  MISC_FEATURE (48)..(48): X= Q, G, R, H or E
  MISC_FEATURE (51)..(51): X= S or L
  MISC_FEATURE (52)..(52): X= L, Q or H
  MISC_FEATURE (54)..(54): X= S, F or Y
  MISC_FEATURE (55)..(55): X= G, K, S, N or R
  MISC_FEATURE (56)..(56): X= D, H, S or N
  MISC_FEATURE (57)..(57): X= A, H, M, E, G, S or T
  MISC_FEATURE (58)..(58): X= S, V, P, T, N or D
  MISC_FEATURE (59)..(59): X= I or L
  MISC_FEATURE (60)..(60): X=  H, S, K, N, Y or E
  MISC_FEATURE (61)..(61): X=  D or E
  MISC_FEATURE (62)..(62): X=  T, I or A
  MISC_FEATURE (63)..(63): X=  V or I
  MISC_FEATURE (64)..(64): X=  E, T, Q, R or K
  MISC_FEATURE (66)..(66): X=  L or V
  MISC_FEATURE (67)..(67): X= I, T or L
  MISC_FEATURE (68)..(68): X=I, M, F, Y or L
  MISC_FEATURE (72)..(72): X= N, T, R, D or S
  MISC_FEATURE (73)..(73): X= S, N, R, T or I
  MISC_FEATURE (75)..(75): X= S or N
  MISC_FEATURE (76)..(76): X= S or A
  MISC_FEATURE (77)..(77): X= N, I or K
  MISC_FEATURE (78)..(78): X= G, E or K
  MISC_FEATURE (79)..(79): X= N, Y, D or T
  MISC_FEATURE (80)..(80): X= V, K or I
  MISC_FEATURE (81)..(81): X= T, A or I
  MISC_FEATURE (83)..(83): X= S, L or T
  MISC_FEATURE (87)..(87): X= E or V
  MISC_FEATURE (93)..(93): X= E or K
  MISC_FEATURE (94)..(94): X= K or R
  MISC_FEATURE (95)..(95): X= N, T or S
  MISC_FEATURE (96)..(96): X= I or F
  MISC_FEATURE (97)..(97): X= K, N, A, or T
  MISC_FEATURE (101)..(101): X= Q, K or E
  MISC_FEATURE (104)..(104): X= V, I or K
  MISC_FEATURE (105)..(105): X= H or R
  MISC_FEATURE (112)..(112): X= N or Y
  MISC_FEATURE (113)..(113): X= = T, S, P, L or A
  MISC_FEATURE (114)..(114): X= = S or P
XWXXVXXDLXXIXXLXXXXHXDXTLYTXSXXHPXCKXTXMXCFLLELXVIXXEXXXXXXXXXXXNXXXLANXXLXXXXXXXEXGCKXCEELEXXXXXEFLXSFXXIVQMFIXXX

SEQ ID NO: 2 - protein, 114 aa, Artificial Sequence
  primate uinterleukin 15 consensus sequence
  MISC_FEATURE (1)..(1): X = N or I
  MISC_FEATURE (4)..(4): X = N or D
  MISC_FEATURE (10)..(10): X = K or R
  MISC_FEATURE (11)..(11): X = K or R
  MISC_FEATURE (13)..(13): X = E or Q
  MISC_FEATURE (16)..(16): X = I or T
  MISC_FEATURE (19)..(19): X = M or I
  MISC_FEATURE (30)..(30): X = D or G
  MISC_FEATURE (31)..(31): X = V or I
  MISC_FEATURE (34)..(34): X = S or R
  MISC_FEATURE (52)..(52): X = L or H
  MISC_FEATURE (55)..(55): X = G or N
  MISC_FEATURE (56)..(56): X = D or N
  MISC_FEATURE (57)..(57): X = A or T
  MISC_FEATURE (58)..(58): X = S, N or D
  MISC_FEATURE (60)..(60): X = H or N
  MISC_FEATURE (63)..(63): X = V or I
  MISC_FEATURE (67)..(67): X = I or L
  MISC_FEATURE (72)..(72): X = N or R
  MISC_FEATURE (73)..(73): X =S or I
  MISC_FEATURE (76)..(76): X =S or A
  MISC_FEATURE (79)..(79): X =N or T
  MISC_FEATURE (80)..(80): X =V or I
  MISC_FEATURE (93)..(93): X =E or K
  MISC_FEATURE (112)..(112): X = N or Y
  MISC_FEATURE (113)..(113): X = T or A
XWVXVISDLXXIXDLXQSXHIDATLYTESXXHPXCKVTAMKCFLLELQVISXESXXXXIXDTXENLXILANXXLSXNGXXTESGCKECEELEXKNIKEFLQSFVHIVQMFIXXS

SEQ ID NO: 3 - protein, 114 aa, Homo sapiens
  VARIANT (93)..(93): X= E or K
NWVNVISDLKKIEDLIQSMHIDATLYTESDVHPSCKVTAMKCFLLELQVISLESGDASIHDTVENLIILANNSLSSNGNVTESGCKECEELEXKNIKEFLQSFVHIVQMFINTS

SEQ ID NO: 4 - protein, 61 aa, Artificial Sequence
  mammalian sushi domain consensus sequence
  MISC_FEATURE (3)..(3): X= P or A
  MISC_FEATURE (5)..(5): X= M or V
  MISC_FEATURE (7)..(7): X= V or I
  MISC_FEATURE (13)..(13): X= W, R or Q
  MISC_FEATURE (16)..(16): X= S or N
  MISC_FEATURE (19)..(19): X= L or V
  MISC_FEATURE (20)..(20): X= Y, H or N
  MISC_FEATURE (26)..(26): X= I or V
  MISC_FEATURE (39)..(39): X= S or T
  MISC_FEATURE (41)..(41): X=T or I
  MISC_FEATURE (45)..(45): X=T or I
  MISC_FEATURE (45)..(45): X= L or I
  MISC_FEATURE (48)..(48): X= A or N
  MISC_FEATURE (51)..(51): X= V or A
  MISC_FEATURE (53)..(53): X= H or Y
CPXPXSXEHADIXVKXYSXXSRERYXCNSGFKRKAGTSXLXECVXNKXTNXAXWTTPSLKC

SEQ ID NO: 5 - protein, 64 aa, Artificial Sequence
  enlarged mammalian sushi domain consensus sequence
  MISC_FEATURE (1)..(1): X= T, V or I
  MISC_FEATURE (5)..(5): X= P or A
  MISC_FEATURE (7)..(7): X= M or V
  MISC_FEATURE (9)..(9): X= V or I
  MISC_FEATURE (15)..(15): X= W, R or Q
  MISC_FEATURE (18)..(18): X= S or N
  MISC_FEATURE (21)..(21): X=L or V
  MISC_FEATURE (22)..(22): X=Y, H or N
  MISC_FEATURE (28)..(28): X= I or V
  MISC_FEATURE (41)..(41): X= S or T
  MISC_FEATURE (43)..(43): X= T or I
  MISC_FEATURE (47)..(47): X= L or I
  MISC_FEATURE (50)..(50): X= A or N
  MISC_FEATURE (53)..(53): X= V or A
  MISC_FEATURE (55)..(55): X= H or Y
XTCPXPXSXEHADIXVKXYSXXSRERYXCNSGFKRKAGTSXLXECVXNKXTNXAXWTTPSLKCI

SEQ ID NO: 6 - protein, 61 aa, Artificial Sequence
  primate sushi domain consensus sequence
  MISC_FEATURE (3)..(3): X= P or A
  MISC_FEATURE (5)..(5): X= M or V
  MISC_FEATURE (13)..(13): X= W, R or Q
  MISC_FEATURE (20)..(20): X= Y or H
  MISC_FEATURE (26)..(26): X= I or V
  MISC_FEATURE (51)..(51): X= V or A
  MISC_FEATURE (53)..(53): X= V or A
CPXPXSVEHADIXVKSYSLXSRERYXCNSGFKRKAGTSSLTECVLNKATNXAXWTTPSLKC

SEQ ID NO: 7 - protein, 63 aa, Artificial Sequence
  enlarged primate sushi domain consensus sequence
  MISC_FEATURE (1)..(1): X= V or I
  MISC_FEATURE (5)..(5): X= P or A
  MISC_FEATURE (7)..(7): X= M or V
  MISC_FEATURE (15)..(15): X= W, R or Q
  MISC_FEATURE (22)..(22): X= Y or H
  MISC_FEATURE (28)..(28): X= I or V
  MISC_FEATURE (53)..(53): X=V or A
  MISC_FEATURE (55)..(55): X=H or Y
XTCPXPXSVEHADIXVKSYSLXSRERYXCNSGFKRKAGTSSLTECVLNKATNXAXWTTPSLKC

SEQ ID NO: 8 - protein, 61 aa, Homo sapiens
CPPPMSVEHADIWVKSYSLYSRERYICNSGFKRKAGTSSLTECVLNKATNVAHWTTPSLKC

SEQ ID NO: 9 - protein, 64 aa, Homo sapiens
ITCPPPMSVEHADIWVKSYSLYSRERYICNSGFKRKAGTSSLTECVLNKATNVAHWTTPSLKCI

SEQ ID NO: 10 - protein, 77 aa, Artificial Sequence
  mammalian sushi and domains consensus sequence
  MISC_FEATURE (1)..(1): X= T, V or I
  MISC_FEATURE (5)..(5): X= P or A
  MISC_FEATURE (7)..(7): X= M or V
  MISC_FEATURE (9)..(9): X= V or I
  MISC_FEATURE (15)..(15): X= W, R or Q
  MISC_FEATURE (18)..(18): X= S or N
  MISC_FEATURE (21)..(21): X= L or V
  MISC_FEATURE (22)..(22): X= Y, H or N
  MISC_FEATURE (28)..(28): X= I or V
  MISC_FEATURE (41)..(41): X= S or T
  MISC_FEATURE (43)..(43): X= T or I
  MISC_FEATURE (47)..(47): X= L or I
  MISC_FEATURE (50)..(50): X=A or N
  MISC_FEATURE (53)..(53): X= V or A
  MISC_FEATURE (55)..(55): X= H or Y
  MISC_FEATURE (55)..(55): X= H or Y
  MISC_FEATURE (68)..(68): X=A, S or L
  MISC_FEATURE (70)..(70): X= V, A, S or T
  MISC_FEATURE (71)..(71): X= H or R
  MISC_FEATURE (72)..(72): X= Q or H
  MISC_FEATURE (73)..(73): X= R, S or K
  MISC_FEATURE (75)..(75): X= A, V or P
  MISC_FEATURE (76)..(76): X= P or S
  MISC_FEATURE (77)..(77): X= P or T
XTCPXPXSXEHADIXVKXYSXXSRERYXCNSGFKRKAGTSXLXECVXNKXTNXAXWTTPSLKCIRDPXLXXXXPXXX

SEQ ID NO: 11 - protein, 77 aa, Artificial Sequence
  primate sushi and domains consensus sequence
  MISC_FEATURE (1)..(1): X= V or I
  MISC_FEATURE (5)..(5): X= P or A
  MISC_FEATURE (7)..(7): X= M or V
  MISC_FEATURE (15)..(15): X= W, R or Q
  MISC_FEATURE (22)..(22): X= Y or H
  MISC_FEATURE (28)..(28): X= I or V
  MISC_FEATURE (53)..(53): X= V or A
  MISC_FEATURE (55)..(55): X= H or Y
  MISC_FEATURE (68)..(68): X= A, S or L
  MISC_FEATURE (70)..(70): X= V, A or T
  MISC_FEATURE (71)..(71): X= H or R
  MISC_FEATURE (75)..(75): X= A or V
XTCPXPXSVEHADIXVKSYSLXSRERYXCNSGFKRKAGTSSLTECVLNKATNXAXWTTPSLKCIRDPXLXXQRPXPP

SEQ ID NO: 12 - protein, 77 aa, Homo sapiens
ITCPPPMSVEHADIWVKSYSLYSRERYICNSGFKRKAGTSSLTECVLNKATNVAHWTTPSLKCIRDPALVHQRPAPP

SEQ ID NO: 13 - protein, 20 aa, Artificial Sequence
  peptidic linker
SGGSGGGGSGGGSGGGGSLQ

SEQ ID NO: 14 - protein, 20 aa, Artificial Sequence
  peptidic linker
SGGSGGGGSGGGSGGGGSGG

SEQ ID NO: 15 - protein, 21 aa, Artificial Sequence
  peptidic linker
SGGGSGGGGSGGGGSGGGSLQ

SEQ ID NO: 16 - protein, 22 aa, Artificial Sequence
  peptidic linker
SGGGGSGGGGSGGGGSGGGGSG

SEQ ID NO: 17 - protein, 22 aa, Artificial Sequence
  peptidic linker
AAGGGSGGGSGGGGSGGGGSAA

SEQ ID NO: 18 - protein, 211 aa, Artificial Sequence
  RLI1
ITCPPPMSVEHADIWVKSYSLYSRERYICNSGFKRKAGTSSLTECVLNKATNVAHWTTPSLKCIRDPALVHQRPAPPSGGSGGGGSGGGSGGGGSLQNWVNVISDLKKIEDLIQSMHIDATLYTESDVHPSCKVTAMKCFLLELQVISLESGDASIHDTVENLIILANNSLSSNGNVTESGCKECEELEEKNIKEFLQSFVHIVQMFINTS

SEQ ID NO: 19 - protein, 211 aa, Artificial Sequence
  RLI2
ITCPPPMSVEHADIWVKSYSLYSRERYICNSGFKRKAGTSSLTECVLNKATNVAHWTTPSLKCIRDPALVHQRPAPPSGGSGGGGSGGGSGGGGSGGNWVNVISDLKKIEDLIQSMHIDATLYTESDVHPSCKVTAMKCFLLELQVISLESGDASIHDTVENLIILANNSLSSNGNVTESGCKECEELEEKNIKEFLQSFVHIVQMFINTS